European Patent Application EP 4 682 165 A1, published January 21, 2026. Title: ＨＰＶ特異的細胞傷害性Ｔ細胞のＴ細胞受容体又はその機能的断片. Applicant: 学校法人順天堂. The sequence listing filed with the application follows.

SEQUENCE LISTING (12 sequences)

SEQ ID NO: 1 - protein, 21 aa, synthetic construct
MKSLRVLLVILWLQLSWVWSQ

SEQ ID NO: 2 - protein, 88 aa, synthetic construct
QKEVEQNSGPLSVPEGAIASLNCTYSDRGSQSFFWYRQYSGKSPELIMFIYSNGDKEDGRFTAQLNKASQYVSLLIRDSQPSDSATYL

SEQ ID NO: 3 - protein, 13 aa, synthetic construct
CAVNGGFGNVLHC

SEQ ID NO: 4 - protein, 10 aa, synthetic construct
GSGTQVIVLP

SEQ ID NO: 5 - protein, 132 aa, synthetic construct
MKSLRVLLVILWLQLSWVWSQQKEVEQNSGPLSVPEGAIASLNCTYSDRGSQSFFWYRQYSGKSPELIMFIYSNGDKEDGRFTAQLNKASQYVSLLIRDSQPSDSATYLCAVNGGFGNVLHCGSGTQVIVLP

SEQ ID NO: 6 - protein, 19 aa, synthetic construct
MGPGLLCWALLCLLGAGLV

SEQ ID NO: 7 - protein, 90 aa, synthetic construct
DAGVTQSPTHLIKTRGQQVTLRCSPKSGHDTVSWYQQALGQGPQFIFQYYEEEERQRGNFPDRFSGHQFPNYSSELNVNALLLGDSALYL

SEQ ID NO: 8 - protein, 15 aa, synthetic construct
CASSLGRAGNQPQHF

SEQ ID NO: 9 - protein, 9 aa, synthetic construct
GDGTRLSIL

SEQ ID NO: 10 - protein, 133 aa, synthetic construct
MGPGLLCWALLCLLGAGLVDAGVTQSPTHLIKTRGQQVTLRCSPKSGHDTVSWYQQALGQGPQFIFQYYEEEERQRGNFPDRFSGHQFPNYSSELNVNALLLGDSALYLCASSLGRAGNQPQHFGDGTRLSIL

SEQ ID NO: 11 - DNA, 396 bp, synthetic construct
  source 1..396: mol_type = other DNA
atgaaatccttgagagttttactagtgatcctgtggcttcagttgagctgggtttggagccaacagaaggaggtggagcagaattctggacccctcagtgttccagagggagccattgcctctctcaactgcacttacagtgaccgaggttcccagtccttcttctggtacagacaatattctgggaaaagccctgagttgataatgttcatatactccaatggtgacaaagaagatggaaggtttacagcacagctcaataaagccagccagtatgtttctctgctcatcagagactcccagcccagtgattcagccacctacctctgtgccgtgaacgggggctttgggaatgtgctgcattgcgggtccggcactcaagtgattgttttacca

SEQ ID NO: 12 - DNA, 399 bp, synthetic construct
  source 1..399: mol_type = other DNA
atgggccccgggctcctctgctgggcactgctttgtctcctgggagcaggcttagtggacgctggagtcacccaaagtcccacacacctgatcaaaacgagaggacagcaagtgactctgagatgctctcctaagtctgggcatgacactgtgtcctggtaccaacaggccctgggtcaggggccccagtttatctttcagtattatgaggaggaagagagacagagaggcaacttccctgatcgattctcaggtcaccagttccctaactatagctctgagctgaatgtgaacgccttgttgctgggggactcggccctctatctctgtgccagcagcttgggacgggcgggcaatcagccccagcattttggtgatgggactcgactctccatccta